European Patent Application EP 4 635 971 A1, published October 22, 2025. Title: synthetic peptide and construct. Applicant: TOAGOSEI CO., LTD. The sequence listing filed with the application follows.

SEQUENCE LISTING (6 sequences)

SEQ ID NO: 1 - protein, 5 aa, synthetic construct
SASAG

SEQ ID NO: 2 - protein, 7 aa, synthetic construct
SASASAG

SEQ ID NO: 3 - protein, 9 aa, synthetic construct
SASASASAG

SEQ ID NO: 4 - protein, 4 aa, synthetic construct
SASA

SEQ ID NO: 5 - protein, 6 aa, synthetic construct
SASASA

SEQ ID NO: 6 - protein, 8 aa, synthetic construct
SASASASA